European Patent Specification EP 3 559 048 B1, published August 12, 2026. Title: Methods for Producing Fabs and IgG Bispecific Antibodies. Applicant: Eli Lilly and Company. The sequence listing filed with the application follows.

SEQUENCE LISTING (84 sequences)

SEQ ID NO: 1 - protein, 337 aa, Artificial Sequence
  Synthetic Construct
ASTKGPSVFPLAPSSKSTSGGTAALGCLVKDYFPEPVTVSWNSGALTSGVHTFPAVLQSSGLYSLSSVVTVPSSSLGTQTYICNVNHKPSNTKVDKKVEPKSCDKGSIEGRGSTHTCPPCPAPELLGGPSVFLFPPKPKDTLMISRTPEVTCVVVDVSHEDPEVKFNWYVDGVEVHNAKTKPREEQYNSTYRVVSVLTVLHQDWLNGKEYKCKVSNKALPAPIEKTISKAKGQPREPQVYTLPPSRDELTKNQVSLTCLVKGFYPSDIAVEWESNGQPENNYKTTPPVLDSDGSFFLYSKLTVDKSRWQQGNVFSCSVMHEALHNHYTQKSLSLSPG

SEQ ID NO: 2 - protein, 107 aa, Artificial Sequence [sequence omitted]

SEQ ID NO: 3 - protein, 122 aa, Artificial Sequence
  Synthetic Construct
HHHHHHHHGGGGSTGRTVAAPSVFIFPPSDEQLKSGTASVVCLLNNFYPREAKVQWKVDNALQSGNSQESVTEQDSKDSTYSLSSTLTLSKADYEKHKVYACEVTHQGLSSPVTKSFNRGEC

SEQ ID NO: 4 - protein, 448 aa, Artificial Sequence
  Synthetic Construct
EVQLVESGGGLVQPGGSLRLSCAASGYTFTSYWLHWVRKAPGKGLEWVGMIDPSNSDTRFNPEFKDRFTISADTSKNTAYLQMNSLRAEDTAVYYCATYRSYVTPLDYWGQGTLVTVSSASTKGPSVFPLAPSSKSTSGGTAALGCLVKDYFPEPVTVSWNSGALTSGVHTFPAVLQSSGLYSLSSVVTVPSSSLGTQTYICNVNHKPSNTKVDKKVEPKSCDKTHTCPPCPAPELLGGPSVFLFPPKPKDTLMISRTPEVTCVVVDVSHEDPEVKFNWYVDGVEVHNAKTKPREEQYQSTYRVVSVLTVLHQDWLNGKEYKCKVSNKALPAPIEKTISKAKGQPREPQVYTLPPSREEMTDNQVSLTCLVKGFYPSDIAVEWESNGQPENNYKTTPPVLMSDGSFFLASKLTVDKSRWQQGNVFSCSVMHEALHNHYTQKSLSLSPG

SEQ ID NO: 5 - protein, 448 aa, Artificial Sequence
  Synthetic Construct
EVQLVESGGGLVQPGGSLRLSCAASGYTFTSYWLHWVRKAPGKGLEWVGMIDPSNSDTRFNPEFKDRFTISADTSKNTAYLQMNSLRAEDTAVYYCATYRSYVTPLDYWGQGTLVTVSSASTKGPSVFPLAPSSKSTSGGTAALGCLVADYFPEPVTVSWNSGALTSGVHTFPAVLQSSGLYSLSSVVTVPSSSLGTQTYICNVNHKPSNTKVDEKVEPKSCDKTHTCPPCPAPELLGGPSVFLFPPKPKDTLMISRTPEVTCVVVDVSHEDPEVKFNWYVDGVEVHNAKTKPREEQYQSTYRVVSVLTVLHQDWLNGKEYKCKVSNKALPAPIEKTISKAKGQPREPQVYTLPPSREEMTDNQVSLTCLVKGFYPSDIAVEWESNGQPENNYKTTPPVLMSDGSFFLASKLTVDKSRWQQGNVFSCSVMHEALHNHYTQKSLSLSPG

SEQ ID NO: 6 - protein, 448 aa, Artificial Sequence
  Synthetic Construct
EVQLVESGGGLVQPGGSLRLSCAASGYTFTSYWLHWVRKAPGKGLEWVGMIDPSNSDTRFNPEFKDRFTISADTSKNTAYLQMNSLRAEDTAVYYCATYRSYVTPLDYWGQGTLVTVSSASTKGPSVFPLAPSSKSTSGGTAALGCLVADYFPEPVTVSWNSGALTSGVHTFPAVLQSSGLYSLASVVTVPSSSLGTQTYICNVNHKPSNTKVDKKVEPKSCDKTHTCPPCPAPELLGGPSVFLFPPKPKDTLMISRTPEVTCVVVDVSHEDPEVKFNWYVDGVEVHNAKTKPREEQYQSTYRVVSVLTVLHQDWLNGKEYKCKVSNKALPAPIEKTISKAKGQPREPQVYTLPPSREEMTDNQVSLTCLVKGFYPSDIAVEWESNGQPENNYKTTPPVLMSDGSFFLASKLTVDKSRWQQGNVFSCSVMHEALHNHYTQKSLSLSPG

SEQ ID NO: 7 - protein, 448 aa, Artificial Sequence
  Synthetic Construct
EVQLVESGGGLVQPGGSLRLSCAASGYTFTSYWLHWVRKAPGKGLEWVGMIDPSNSDTRFNPEFKDRFTISADTSKNTAYLQMNSLRAEDTAVYYCATYRSYVTPLDYWGQGTLVTVSSASTKGPSVFPLAPSSKSTSGGTAALGCLVADYFPEPVTVSWNSGALTSGVHTFPAVLQSSGLYSLGSVVTVPSSSLGTQTYICNVNHKPSNTKVDKKVEPKSCDKTHTCPPCPAPELLGGPSVFLFPPKPKDTLMISRTPEVTCVVVDVSHEDPEVKFNWYVDGVEVHNAKTKPREEQYQSTYRVVSVLTVLHQDWLNGKEYKCKVSNKALPAPIEKTISKAKGQPREPQVYTLPPSREEMTDNQVSLTCLVKGFYPSDIAVEWESNGQPENNYKTTPPVLMSDGSFFLASKLTVDKSRWQQGNVFSCSVMHEALHNHYTQKSLSLSPG

SEQ ID NO: 8 - protein, 448 aa, Artificial Sequence
  Synthetic Construct
EVQLVESGGGLVQPGGSLRLSCAASGYTFTSYWLHWVRKAPGKGLEWVGMIDPSNSDTRFNPEFKDRFTISADTSKNTAYLQMNSLRAEDTAVYYCATYRSYVTPLDYWGQGTLVTVSSASTKGPSVFPLAPSSKSTSGGTAALGCLVADYFPEPVTVSWNSGALTSGVHTFPAVLQSSGLYSLASVVTVPSSSLGTQTYICNVNHKPSNTKVDEKVEPKSCDKTHTCPPCPAPELLGGPSVFLFPPKPKDTLMISRTPEVTCVVVDVSHEDPEVKFNWYVDGVEVHNAKTKPREEQYQSTYRVVSVLTVLHQDWLNGKEYKCKVSNKALPAPIEKTISKAKGQPREPQVYTLPPSREEMTDNQVSLTCLVKGFYPSDIAVEWESNGQPENNYKTTPPVLMSDGSFFLASKLTVDKSRWQQGNVFSCSVMHEALHNHYTQKSLSLSPG

SEQ ID NO: 9 - protein, 448 aa, Artificial Sequence
  Synthetic Construct
EVQLVESGGGLVQPGGSLRLSCAASGYTFTSYWLHWVRKAPGKGLEWVGMIDPSNSDTRFNPEFKDRFTISADTSKNTAYLQMNSLRAEDTAVYYCATYRSYVTPLDYWGQGTLVTVSSASTKGPSVFPLAPSSKSTSGGTAALGCLVADYFPEPVTVSWNSGALTSGVHTFPAVLQSSGLYSLGSVVTVPSSSLGTQTYICNVNHKPSNTKVDEKVEPKSCDKTHTCPPCPAPELLGGPSVFLFPPKPKDTLMISRTPEVTCVVVDVSHEDPEVKFNWYVDGVEVHNAKTKPREEQYQSTYRVVSVLTVLHQDWLNGKEYKCKVSNKALPAPIEKTISKAKGQPREPQVYTLPPSREEMTDNQVSLTCLVKGFYPSDIAVEWESNGQPENNYKTTPPVLMSDGSFFLASKLTVDKSRWQQGNVFSCSVMHEALHNHYTQKSLSLSPG

SEQ ID NO: 10 - protein, 220 aa, Artificial Sequence
  Synthetic Construct
RIQMTQSPSSLSASVGDRVTITCKSSQSLLYTSSQKNYLAWYQDKPGKAPKLLIYWASTRESGVPSRFSGSGSGTDFTLTISSLQPEDFATYYCQQYYAYPWTFGQGTKVEIKRTVAAPSVFIFPPSDEQLKSGTASVVCLLNNFYPREAKVQWKVDNALQSGNSQESVTEQDSKDSTYSLSSTLTLSKADYEKHKVYACEVTHQGLSSPVTKSFNRGEC

SEQ ID NO: 11 - protein, 220 aa, Artificial Sequence
  Synthetic Construct
RIQMTQSPSSLSASVGDRVTITCKSSQSLLYTSSQKNYLAWYQDKPGKAPKLLIYWASTRESGVPSRFSGSGSGTDFTLTISSLQPEDFATYYCQQYYAYPWTFGQGTKVEIKRTVAAPSVFIFPPSDKQLKSGTARVVCLLNNFYPREAKVQWKVDNALQSGNSQESVTEQDSKDSTYSLSSTLTLSKADYEKHKVYACEVTHQGLSSPVTKSFNRGEC

SEQ ID NO: 12 - protein, 220 aa, Artificial Sequence
  Synthetic Construct
RIQMTQSPSSLSASVGDRVTITCKSSQSLLYTSSQKNYLAWYQDKPGKAPKLLIYWASTRESGVPSRFSGSGSGTDFTLTISSLQPEDFATYYCQQYYAYPWTFGQGTKVEIKRTVAAPSVFIFPPSDEQLKSGTARVVCLLNNFYPREAKVQWKVDNALQSGNSQESVTEQDSKDSTYSLISTLTLSKADYEKHKVYACEVTHQGLSSPVTKSFNRGEC

SEQ ID NO: 13 - protein, 220 aa, Artificial Sequence
  Synthetic Construct
RIQMTQSPSSLSASVGDRVTITCKSSQSLLYTSSQKNYLAWYQDKPGKAPKLLIYWASTRESGVPSRFSGSGSGTDFTLTISSLQPEDFATYYCQQYYAYPWTFGQGTKVEIKRTVAAPSVFIFPPSDKQLKSGTARVVCLLNNFYPREAKVQWKVDNALQSGNSQESVTEQDSKDSTYSLISTLTLSKADYEKHKVYACEVTHQGLSSPVTKSFNRGEC

SEQ ID NO: 14 - protein, 448 aa, Artificial Sequence
  Synthetic Construct
EVQLVESGGGLVQPGGSLRLSCAASGFTFTDYTMDWVRKAPGKGLEWVADVNPNSGGSIYNQEFKGRFTLSVDRSKNTLYLQMNSLRAEDTAVYYCARNLGPSFYFDYWGQGTLVTVSSASTKGPSVFPLAPSSKSTSGGTAALGCLVKDYFPEPVTVSWNSGALTSGVHTFPAVLQSSGLYSLSSVVTVPSSSLGTQTYICNVNHKPSNTKVDKKVEPKSCDKTHTCPPCPAPELLGGPSVFLFPPKPKDTLMISRTPEVTCVVVDVSHEDPEVKFNWYVDGVEVHNAKTKPREEQYQSTYRVVSVLTVLHQDWLNGKEYKCKVSNKALPAPIEKTISKAKGQPREPQVYTLPPSREEMTDNQVSLTCLVKGFYPSDIAVEWESNGQPENNYKTTPPVLMSDGSFFLASKLTVDKSRWQQGNVFSCSVMHEALHNHYTQKSLSLSPG

SEQ ID NO: 15 - protein, 448 aa, Artificial Sequence
  Synthetic Construct
EVQLVESGGGLVQPGGSLRLSCAASGFTFTDYTMDWVRKAPGKGLEWVADVNPNSGGSIYNQEFKGRFTLSVDRSKNTLYLQMNSLRAEDTAVYYCARNLGPSFYFDYWGQGTLVTVSSASTKGPSVFPLAPSSKSTSGGTAALGCLVADYFPEPVTVSWNSGALTSGVHTFPAVLQSSGLYSLSSVVTVPSSSLGTQTYICNVNHKPSNTKVDEKVEPKSCDKTHTCPPCPAPELLGGPSVFLFPPKPKDTLMISRTPEVTCVVVDVSHEDPEVKFNWYVDGVEVHNAKTKPREEQYQSTYRVVSVLTVLHQDWLNGKEYKCKVSNKALPAPIEKTISKAKGQPREPQVYTLPPSREEMTDNQVSLTCLVKGFYPSDIAVEWESNGQPENNYKTTPPVLMSDGSFFLASKLTVDKSRWQQGNVFSCSVMHEALHNHYTQKSLSLSPG

SEQ ID NO: 16 - protein, 448 aa, Artificial Sequence
  Synthetic Construct
EVQLVESGGGLVQPGGSLRLSCAASGFTFTDYTMDWVRKAPGKGLEWVADVNPNSGGSIYNQEFKGRFTLSVDRSKNTLYLQMNSLRAEDTAVYYCARNLGPSFYFDYWGQGTLVTVSSASTKGPSVFPLAPSSKSTSGGTAALGCLVADYFPEPVTVSWNSGALTSGVHTFPAVLQSSGLYSLASVVTVPSSSLGTQTYICNVNHKPSNTKVDKKVEPKSCDKTHTCPPCPAPELLGGPSVFLFPPKPKDTLMISRTPEVTCVVVDVSHEDPEVKFNWYVDGVEVHNAKTKPREEQYQSTYRVVSVLTVLHQDWLNGKEYKCKVSNKALPAPIEKTISKAKGQPREPQVYTLPPSREEMTDNQVSLTCLVKGFYPSDIAVEWESNGQPENNYKTTPPVLMSDGSFFLASKLTVDKSRWQQGNVFSCSVMHEALHNHYTQKSLSLSPG

SEQ ID NO: 17 - protein, 448 aa, Artificial Sequence
  Synthetic Construct
EVQLVESGGGLVQPGGSLRLSCAASGFTFTDYTMDWVRKAPGKGLEWVADVNPNSGGSIYNQEFKGRFTLSVDRSKNTLYLQMNSLRAEDTAVYYCARNLGPSFYFDYWGQGTLVTVSSASTKGPSVFPLAPSSKSTSGGTAALGCLVADYFPEPVTVSWNSGALTSGVHTFPAVLQSSGLYSLGSVVTVPSSSLGTQTYICNVNHKPSNTKVDKKVEPKSCDKTHTCPPCPAPELLGGPSVFLFPPKPKDTLMISRTPEVTCVVVDVSHEDPEVKFNWYVDGVEVHNAKTKPREEQYQSTYRVVSVLTVLHQDWLNGKEYKCKVSNKALPAPIEKTISKAKGQPREPQVYTLPPSREEMTDNQVSLTCLVKGFYPSDIAVEWESNGQPENNYKTTPPVLMSDGSFFLASKLTVDKSRWQQGNVFSCSVMHEALHNHYTQKSLSLSPG

SEQ ID NO: 18 - protein, 448 aa, Artificial Sequence
  Synthetic Construct
EVQLVESGGGLVQPGGSLRLSCAASGFTFTDYTMDWVRKAPGKGLEWVADVNPNSGGSIYNQEFKGRFTLSVDRSKNTLYLQMNSLRAEDTAVYYCARNLGPSFYFDYWGQGTLVTVSSASTKGPSVFPLAPSSKSTSGGTAALGCLVADYFPEPVTVSWNSGALTSGVHTFPAVLQSSGLYSLASVVTVPSSSLGTQTYICNVNHKPSNTKVDEKVEPKSCDKTHTCPPCPAPELLGGPSVFLFPPKPKDTLMISRTPEVTCVVVDVSHEDPEVKFNWYVDGVEVHNAKTKPREEQYQSTYRVVSVLTVLHQDWLNGKEYKCKVSNKALPAPIEKTISKAKGQPREPQVYTLPPSREEMTDNQVSLTCLVKGFYPSDIAVEWESNGQPENNYKTTPPVLMSDGSFFLASKLTVDKSRWQQGNVFSCSVMHEALHNHYTQKSLSLSPG

SEQ ID NO: 19 - protein, 448 aa, Artificial Sequence
  Synthetic Construct
EVQLVESGGGLVQPGGSLRLSCAASGFTFTDYTMDWVRKAPGKGLEWVADVNPNSGGSIYNQEFKGRFTLSVDRSKNTLYLQMNSLRAEDTAVYYCARNLGPSFYFDYWGQGTLVTVSSASTKGPSVFPLAPSSKSTSGGTAALGCLVADYFPEPVTVSWNSGALTSGVHTFPAVLQSSGLYSLGSVVTVPSSSLGTQTYICNVNHKPSNTKVDEKVEPKSCDKTHTCPPCPAPELLGGPSVFLFPPKPKDTLMISRTPEVTCVVVDVSHEDPEVKFNWYVDGVEVHNAKTKPREEQYQSTYRVVSVLTVLHQDWLNGKEYKCKVSNKALPAPIEKTISKAKGQPREPQVYTLPPSREEMTDNQVSLTCLVKGFYPSDIAVEWESNGQPENNYKTTPPVLMSDGSFFLASKLTVDKSRWQQGNVFSCSVMHEALHNHYTQKSLSLSPG

SEQ ID NO: 20 - protein, 214 aa, Artificial Sequence
  Synthetic Construct
RIQMTQSPSSLSASVGDRVTITCKASQDVSIGVAWYQDKPGKAPKLLIYSASYRYTGVPSRFSGSGSGTDFTLTISSLQPEDFATYYCQQYYIYPYTFGQGTKVEIKRTVAAPSVFIFPPSDEQLKSGTASVVCLLNNFYPREAKVQWKVDNALQSGNSQESVTEQDSKDSTYSLSSTLTLSKADYEKHKVYACEVTHQGLSSPVTKSFNRGEC

SEQ ID NO: 21 - protein, 214 aa, Artificial Sequence
  Synthetic Construct
RIQMTQSPSSLSASVGDRVTITCKASQDVSIGVAWYQDKPGKAPKLLIYSASYRYTGVPSRFSGSGSGTDFTLTISSLQPEDFATYYCQQYYIYPYTFGQGTKVEIKRTVAAPSVFIFPPSDKQLKSGTARVVCLLNNFYPREAKVQWKVDNALQSGNSQESVTEQDSKDSTYSLSSTLTLSKADYEKHKVYACEVTHQGLSSPVTKSFNRGEC

SEQ ID NO: 22 - protein, 214 aa, Artificial Sequence
  Synthetic Construct
RIQMTQSPSSLSASVGDRVTITCKASQDVSIGVAWYQDKPGKAPKLLIYSASYRYTGVPSRFSGSGSGTDFTLTISSLQPEDFATYYCQQYYIYPYTFGQGTKVEIKRTVAAPSVFIFPPSDEQLKSGTARVVCLLNNFYPREAKVQWKVDNALQSGNSQESVTEQDSKDSTYSLISTLTLSKADYEKHKVYACEVTHQGLSSPVTKSFNRGEC

SEQ ID NO: 23 - protein, 214 aa, Artificial Sequence
  Synthetic Construct
RIQMTQSPSSLSASVGDRVTITCKASQDVSIGVAWYQDKPGKAPKLLIYSASYRYTGVPSRFSGSGSGTDFTLTISSLQPEDFATYYCQQYYIYPYTFGQGTKVEIKRTVAAPSVFIFPPSDKQLKSGTARVVCLLNNFYPREAKVQWKVDNALQSGNSQESVTEQDSKDSTYSLISTLTLSKADYEKHKVYACEVTHQGLSSPVTKSFNRGEC

SEQ ID NO: 24 - protein, 450 aa, Artificial Sequence
  Synthetic Construct
QVQLVQSGAEVKKPGASVKVSCKASGYTFTSHWMHWVRYAPGQGLEWIGEFNPSNGRTNYNEKFKSKATMTVDTSTNTAYMELSSLRSEDTAVYYCASRDYDYDGRYFDYWGRGTLVTVSSASTKGPSVFPLAPSSKSTSGGTAALGCLVKDYFPEPVTVSWNSGALTSGVHTFPAVLQSSGLYSLSSVVTVPSSSLGTQTYICNVNHKPSNTKVDKKVEPKSCDKTHTCPPCPAPELLGGPSVFLFPPKPKDTLMISRTPEVTCVVVDVSHEDPEVKFNWYVDGVEVHNAKTKPREEQYQSTYRVVSVLTVLHQDWLNGKEYKCKVSNKALPAPIEKTISKAKGQPRRPRVYTLPPSREEMTKNQVSLVCLVKGFYPSDIAVEWESNGQPENNYKTTPPVLDSDGSFFLYSVLTVDKSRWQQGNVFSCSVMHEALHNHYTQKSLSLSPG

SEQ ID NO: 25 - protein, 450 aa, Artificial Sequence
  Synthetic Construct
QVQLVQSGAEVKKPGASVKVSCKASGYTFTSHWMHWVRYAPGQGLEWIGEFNPSNGRTNYNEKFKSKATMTVDTSTNTAYMELSSLRSEDTAVYYCASRDYDYDGRYFDYWGRGTLVTVSSASTKGPSVFPLAPSSKSTSGGTAALGCLVKDYFPEPVTVSWNSGALTSGVHTFPAVLQSSGLYSLSSVVTVPSSSLGTQTYICNVNHKPSNTKVDEKVEPKSCDKTHTCPPCPAPELLGGPSVFLFPPKPKDTLMISRTPEVTCVVVDVSHEDPEVKFNWYVDGVEVHNAKTKPREEQYQSTYRVVSVLTVLHQDWLNGKEYKCKVSNKALPAPIEKTISKAKGQPRRPRVYTLPPSREEMTKNQVSLVCLVKGFYPSDIAVEWESNGQPENNYKTTPPVLDSDGSFFLYSVLTVDKSRWQQGNVFSCSVMHEALHNHYTQKSLSLSPG

SEQ ID NO: 26 - protein, 213 aa, Artificial Sequence
  Synthetic Construct
DIQMTQSPSSLSASVGDRVTITCSASSSVTYMYWYQRKPGDAPKLLIYDTSNLASGVPSRFSGSGSGTDYTFTISSLQPEDIATYYCQQWSSHIFTFGQGTKVEIKRTVAAPSVFIFPPSDEQLKSGTASVVCLLNNFYPREAKVQWKVDNALQSGNSQESVTEQDSKDSTYSLSSTLTLSKADYEKHKVYACEVTHQGLSSPVTKSFNRGEC

SEQ ID NO: 27 - protein, 213 aa, Artificial Sequence
  Synthetic Construct
DIQMTQSPSSLSASVGDRVTITCSASSSVTYMYWYQRKPGDAPKLLIYDTSNLASGVPSRFSGSGSGTDYTFTISSLQPEDIATYYCQQWSSHIFTFGQGTKVEIKRTVAAPSVFIFPPSDKQLKSGTASVVCLLNNFYPREAKVQWKVDNALQSGNSQESVTEQDSKDSTYSLSSTLTLSKADYEKHKVYACEVTHQGLSSPVTKSFNRGEC

SEQ ID NO: 28 - protein, 445 aa, Artificial Sequence
  Synthetic Construct
QVQLVQSGAEVKKPGSSVKVSCKASGYTFTTYYLHWVRYAPGQGLEWMGWIYPGNVHAQYNEKFKGRVTITADKSTSTAYMELSSLRSEDTAVYYCARSWEGFPYWGRGTTVTVSSASTKGPSVFPLAPSSKSTSGGTAALGCLVKDYFPEPVTVSWNSGALTSGVHTFPAVLQSSGLYSLSSVVTVPSSSLGTQTYICNVNHKPSNTKVDKKVEPKSCDKTHTCPPCPAPELLGGPSVFLFPPKPKDTLMISRTPEVTCVVVDVSHEDPEVKFNWYVDGVEVHNAKTKPREEQYQSTYRVVSVLTVLHQDWLNGKEYKCKVSNKALPAPIEKTISKAKGQPRRPRVYTLPPSREEMTKNQVSLVCLVKGFYPSDIAVEWESNGQPENNYKTTPPVLDSDGSFFLYSVLTVDKSRWQQGNVFSCSVMHEALHNHYTQKSLSLSPG

SEQ ID NO: 29 - protein, 445 aa, Artificial Sequence
  Synthetic Construct
QVQLVQSGAEVKKPGSSVKVSCKASGYTFTTYYLHWVRYAPGQGLEWMGWIYPGNVHAQYNEKFKGRVTITADKSTSTAYMELSSLRSEDTAVYYCARSWEGFPYWGRGTTVTVSSASTKGPSVFPLAPSSKSTSGGTAALGCLVKDYFPEPVTVSWNSGALTSGVHTFPAVLQSSGLYSLSSVVTVPSSSLGTQTYICNVNHKPSNTKVDEKVEPKSCDKTHTCPPCPAPELLGGPSVFLFPPKPKDTLMISRTPEVTCVVVDVSHEDPEVKFNWYVDGVEVHNAKTKPREEQYQSTYRVVSVLTVLHQDWLNGKEYKCKVSNKALPAPIEKTISKAKGQPRRPRVYTLPPSREEMTKNQVSLVCLVKGFYPSDIAVEWESNGQPENNYKTTPPVLDSDGSFFLYSVLTVDKSRWQQGNVFSCSVMHEALHNHYTQKSLSLSPG

SEQ ID NO: 30 - protein, 214 aa, Artificial Sequence
  Synthetic Construct
DIQMTQSPSSLSASVGDRVTITCKASQNVGINVAWYQRKPGDAPKSLISSASYRYSGVPSRFSGSGSGTDFTLTISSLQPEDFATYFCQQYDTYPFTFGQGTKVEIKRTVAAPSVFIFPPSDEQLKSGTASVVCLLNNFYPREAKVQWKVDNALQSGNSQESVTEQDSKDSTYSLSSTLTLSKADYEKHKVYACEVTHQGLSSPVTKSFNRGEC

SEQ ID NO: 31 - protein, 214 aa, Artificial Sequence
  Synthetic Construct
DIQMTQSPSSLSASVGDRVTITCKASQNVGINVAWYQRKPGDAPKSLISSASYRYSGVPSRFSGSGSGTDFTLTISSLQPEDFATYFCQQYDTYPFTFGQGTKVEIKRTVAAPSVFIFPPSDKQLKSGTASVVCLLNNFYPREAKVQWKVDNALQSGNSQESVTEQDSKDSTYSLSSTLTLSKADYEKHKVYACEVTHQGLSSPVTKSFNRGEC

SEQ ID NO: 32 - protein, 448 aa, Artificial Sequence
  Synthetic Construct
EVQLVESGGGLVQPGGSLRLSCAASGYTFTSYWLHWVRQAPGKGLEWVGMIDPSNSDTRFNPNFKDRFTISADTSKNTAYLQMNSLRAEDTAVYYCATYRSYVTPLDYWGQGTLVTVSSASTKGPSVFPLAPSSKSTSGGTAALGCLVKDYFPEPVTVSWNSGALTSGVHTFPAVLQSSGLYSLSSVVTVPSSSLGTQTYICNVNHKPSNTKVDKKVEPKSCDKTHTCPPCPAPELLGGPSVFLFPPKPKDTLMISRTPEVTCVVVDVSHEDPEVKFNWYVDGVEVHNAKTKPREEQYQSTYRVVSVLTVLHQDWLNGKEYKCKVSNKALPAPIEKTISKAKGQPREPQVYTLPPSREEMTDNQVSLTCLVKGFYPSDIAVEWESNGQPENNYKTTPPVLMSDGSFFLASKLTVDKSRWQQGNVFSCSVMHEALHNHYTQKSLSLSPG

SEQ ID NO: 33 - protein, 448 aa, Artificial Sequence
  Synthetic Construct
EVQLVESGGGLVQPGGSLRLSCAASGYTFTSYWLHWVRQAPGKGLEWVGMIDPSNSDTRFNPNFKDRFTISADTSKNTAYLQMNSLRAEDTAVYYCATYRSYVTPLDYWGQGTLVTVSSASTKGPSVFPLAPSSKSTSGGTAALGCLVADYFPEPVTVSWNSGALTSGVHTFPAVLQSSGLYSLSSVVTVPSSSLGTQTYICNVNHKPSNTKVDEKVEPKSCDKTHTCPPCPAPELLGGPSVFLFPPKPKDTLMISRTPEVTCVVVDVSHEDPEVKFNWYVDGVEVHNAKTKPREEQYQSTYRVVSVLTVLHQDWLNGKEYKCKVSNKALPAPIEKTISKAKGQPREPQVYTLPPSREEMTDNQVSLTCLVKGFYPSDIAVEWESNGQPENNYKTTPPVLMSDGSFFLASKLTVDKSRWQQGNVFSCSVMHEALHNHYTQKSLSLSPG

SEQ ID NO: 34 - protein, 448 aa, Artificial Sequence
  Synthetic Construct
EVQLVESGGGLVQPGGSLRLSCAASGYTFTSYWLHWVRQAPGKGLEWVGMIDPSNSDTRFNPNFKDRFTISADTSKNTAYLQMNSLRAEDTAVYYCATYRSYVTPLDYWGQGTLVTVSSASTKGPSVFPLAPSSKSTSGGTAALGCLVADYFPEPVTVSWNSGALTSGVHTFPAVLQSSGLYSLASVVTVPSSSLGTQTYICNVNHKPSNTKVDKKVEPKSCDKTHTCPPCPAPELLGGPSVFLFPPKPKDTLMISRTPEVTCVVVDVSHEDPEVKFNWYVDGVEVHNAKTKPREEQYQSTYRVVSVLTVLHQDWLNGKEYKCKVSNKALPAPIEKTISKAKGQPREPQVYTLPPSREEMTDNQVSLTCLVKGFYPSDIAVEWESNGQPENNYKTTPPVLMSDGSFFLASKLTVDKSRWQQGNVFSCSVMHEALHNHYTQKSLSLSPG

SEQ ID NO: 35 - protein, 448 aa, Artificial Sequence
  Synthetic Construct
EVQLVESGGGLVQPGGSLRLSCAASGYTFTSYWLHWVRQAPGKGLEWVGMIDPSNSDTRFNPNFKDRFTISADTSKNTAYLQMNSLRAEDTAVYYCATYRSYVTPLDYWGQGTLVTVSSASTKGPSVFPLAPSSKSTSGGTAALGCLVADYFPEPVTVSWNSGALTSGVHTFPAVLQSSGLYSLGSVVTVPSSSLGTQTYICNVNHKPSNTKVDKKVEPKSCDKTHTCPPCPAPELLGGPSVFLFPPKPKDTLMISRTPEVTCVVVDVSHEDPEVKFNWYVDGVEVHNAKTKPREEQYQSTYRVVSVLTVLHQDWLNGKEYKCKVSNKALPAPIEKTISKAKGQPREPQVYTLPPSREEMTDNQVSLTCLVKGFYPSDIAVEWESNGQPENNYKTTPPVLMSDGSFFLASKLTVDKSRWQQGNVFSCSVMHEALHNHYTQKSLSLSPG

SEQ ID NO: 36 - protein, 220 aa, Artificial Sequence
  Synthetic Construct
DIQMTQSPSSLSASVGDRVTITCKSSQSLLYTSSQKNYLAWYQQKPGKAPKLLIYWASTRESGVPSRFSGSGSGTDFTLTISSLQPEDFATYYCQQYYAYPWTFGQGTKVEIKRTVAAPSVFIFPPSDEQLKSGTASVVCLLNNFYPREAKVQWKVDNALQSGNSQESVTEQDSKDSTYSLSSTLTLSKADYEKHKVYACEVTHQGLSSPVTKSFNRGEC

SEQ ID NO: 37 - protein, 220 aa, Artificial Sequence
  Synthetic Construct
DIQMTQSPSSLSASVGDRVTITCKSSQSLLYTSSQKNYLAWYQQKPGKAPKLLIYWASTRESGVPSRFSGSGSGTDFTLTISSLQPEDFATYYCQQYYAYPWTFGQGTKVEIKRTVAAPSVFIFPPSDKQLKSGTARVVCLLNNFYPREAKVQWKVDNALQSGNSQESVTEQDSKDSTYSLSSTLTLSKADYEKHKVYACEVTHQGLSSPVTKSFNRGEC

SEQ ID NO: 38 - protein, 220 aa, Artificial Sequence
  Synthetic Construct
DIQMTQSPSSLSASVGDRVTITCKSSQSLLYTSSQKNYLAWYQQKPGKAPKLLIYWASTRESGVPSRFSGSGSGTDFTLTISSLQPEDFATYYCQQYYAYPWTFGQGTKVEIKRTVAAPSVFIFPPSDEQLKSGTARVVCLLNNFYPREAKVQWKVDNALQSGNSQESVTEQDSKDSTYSLISTLTLSKADYEKHKVYACEVTHQGLSSPVTKSFNRGEC

SEQ ID NO: 39 - protein, 448 aa, Artificial Sequence
  Synthetic Construct
EVQLVESGGGLVQPGGSLRLSCAASGFTFTDYTMDWVRQAPGKGLEWVADVNPNSGGSIYNQRFKGRFTLSVDRSKNTLYLQMNSLRAEDTAVYYCARNLGPSFYFDYWGQGTLVTVSSASTKGPSVFPLAPSSKSTSGGTAALGCLVKDYFPEPVTVSWNSGALTSGVHTFPAVLQSSGLYSLSSVVTVPSSSLGTQTYICNVNHKPSNTKVDKKVEPKSCDKTHTCPPCPAPELLGGPSVFLFPPKPKDTLMISRTPEVTCVVVDVSHEDPEVKFNWYVDGVEVHNAKTKPREEQYQSTYRVVSVLTVLHQDWLNGKEYKCKVSNKALPAPIEKTISKAKGQPREPQVYTLPPSREEMTDNQVSLTCLVKGFYPSDIAVEWESNGQPENNYKTTPPVLMSDGSFFLASKLTVDKSRWQQGNVFSCSVMHEALHNHYTQKSLSLSPG

SEQ ID NO: 40 - protein, 448 aa, Artificial Sequence
  Synthetic Construct
EVQLVESGGGLVQPGGSLRLSCAASGFTFTDYTMDWVRQAPGKGLEWVADVNPNSGGSIYNQRFKGRFTLSVDRSKNTLYLQMNSLRAEDTAVYYCARNLGPSFYFDYWGQGTLVTVSSASTKGPSVFPLAPSSKSTSGGTAALGCLVADYFPEPVTVSWNSGALTSGVHTFPAVLQSSGLYSLSSVVTVPSSSLGTQTYICNVNHKPSNTKVDEKVEPKSCDKTHTCPPCPAPELLGGPSVFLFPPKPKDTLMISRTPEVTCVVVDVSHEDPEVKFNWYVDGVEVHNAKTKPREEQYQSTYRVVSVLTVLHQDWLNGKEYKCKVSNKALPAPIEKTISKAKGQPREPQVYTLPPSREEMTDNQVSLTCLVKGFYPSDIAVEWESNGQPENNYKTTPPVLMSDGSFFLASKLTVDKSRWQQGNVFSCSVMHEALHNHYTQKSLSLSPG

SEQ ID NO: 41 - protein, 448 aa, Artificial Sequence
  Synthetic Construct
EVQLVESGGGLVQPGGSLRLSCAASGFTFTDYTMDWVRQAPGKGLEWVADVNPNSGGSIYNQRFKGRFTLSVDRSKNTLYLQMNSLRAEDTAVYYCARNLGPSFYFDYWGQGTLVTVSSASTKGPSVFPLAPSSKSTSGGTAALGCLVADYFPEPVTVSWNSGALTSGVHTFPAVLQSSGLYSLASVVTVPSSSLGTQTYICNVNHKPSNTKVDKKVEPKSCDKTHTCPPCPAPELLGGPSVFLFPPKPKDTLMISRTPEVTCVVVDVSHEDPEVKFNWYVDGVEVHNAKTKPREEQYQSTYRVVSVLTVLHQDWLNGKEYKCKVSNKALPAPIEKTISKAKGQPREPQVYTLPPSREEMTDNQVSLTCLVKGFYPSDIAVEWESNGQPENNYKTTPPVLMSDGSFFLASKLTVDKSRWQQGNVFSCSVMHEALHNHYTQKSLSLSPG

SEQ ID NO: 42 - protein, 448 aa, Artificial Sequence
  Synthetic Construct
EVQLVESGGGLVQPGGSLRLSCAASGFTFTDYTMDWVRQAPGKGLEWVADVNPNSGGSIYNQRFKGRFTLSVDRSKNTLYLQMNSLRAEDTAVYYCARNLGPSFYFDYWGQGTLVTVSSASTKGPSVFPLAPSSKSTSGGTAALGCLVADYFPEPVTVSWNSGALTSGVHTFPAVLQSSGLYSLGSVVTVPSSSLGTQTYICNVNHKPSNTKVDKKVEPKSCDKTHTCPPCPAPELLGGPSVFLFPPKPKDTLMISRTPEVTCVVVDVSHEDPEVKFNWYVDGVEVHNAKTKPREEQYQSTYRVVSVLTVLHQDWLNGKEYKCKVSNKALPAPIEKTISKAKGQPREPQVYTLPPSREEMTDNQVSLTCLVKGFYPSDIAVEWESNGQPENNYKTTPPVLMSDGSFFLASKLTVDKSRWQQGNVFSCSVMHEALHNHYTQKSLSLSPG

SEQ ID NO: 43 - protein, 214 aa, Artificial Sequence
  Synthetic Construct
DIQMTQSPSSLSASVGDRVTITCKASQDVSIGVAWYQQKPGKAPKLLIYSASYRYTGVPSRFSGSGSGTDFTLTISSLQPEDFATYYCQQYYIYPYTFGQGTKVEIKRTVAAPSVFIFPPSDEQLKSGTASVVCLLNNFYPREAKVQWKVDNALQSGNSQESVTEQDSKDSTYSLSSTLTLSKADYEKHKVYACEVTHQGLSSPVTKSFNRGEC

SEQ ID NO: 44 - protein, 214 aa, Artificial Sequence
  Synthetic Construct
DIQMTQSPSSLSASVGDRVTITCKASQDVSIGVAWYQQKPGKAPKLLIYSASYRYTGVPSRFSGSGSGTDFTLTISSLQPEDFATYYCQQYYIYPYTFGQGTKVEIKRTVAAPSVFIFPPSDKQLKSGTARVVCLLNNFYPREAKVQWKVDNALQSGNSQESVTEQDSKDSTYSLSSTLTLSKADYEKHKVYACEVTHQGLSSPVTKSFNRGEC

SEQ ID NO: 45 - protein, 214 aa, Artificial Sequence
  Synthetic Construct
DIQMTQSPSSLSASVGDRVTITCKASQDVSIGVAWYQQKPGKAPKLLIYSASYRYTGVPSRFSGSGSGTDFTLTISSLQPEDFATYYCQQYYIYPYTFGQGTKVEIKRTVAAPSVFIFPPSDEQLKSGTARVVCLLNNFYPREAKVQWKVDNALQSGNSQESVTEQDSKDSTYSLISTLTLSKADYEKHKVYACEVTHQGLSSPVTKSFNRGEC

SEQ ID NO: 46 - protein, 450 aa, Artificial Sequence
  Synthetic Construct
QVQLVQSGAEVKKPGASVKVSCKASGYTFTSHWMHWVRQAPGQGLEWIGEFNPSNGRTNYNEKFKSKATMTVDTSTNTAYMELSSLRSEDTAVYYCASRDYDYDGRYFDYWGQGTLVTVSSASTKGPSVFPLAPSSKSTSGGTAALGCLVKDYFPEPVTVSWNSGALTSGVHTFPAVLQSSGLYSLSSVVTVPSSSLGTQTYICNVNHKPSNTKVDKKVEPKSCDKTHTCPPCPAPELLGGPSVFLFPPKPKDTLMISRTPEVTCVVVDVSHEDPEVKFNWYVDGVEVHNAKTKPREEQYQSTYRVVSVLTVLHQDWLNGKEYKCKVSNKALPAPIEKTISKAKGQPRRPRVYTLPPSREEMTKNQVSLVCLVKGFYPSDIAVEWESNGQPENNYKTTPPVLDSDGSFFLYSVLTVDKSRWQQGNVFSCSVMHEALHNHYTQKSLSLSPG

SEQ ID NO: 47 - protein, 450 aa, Artificial Sequence
  Synthetic Construct
QVQLVQSGAEVKKPGASVKVSCKASGYTFTSHWMHWVRQAPGQGLEWIGEFNPSNGRTNYNEKFKSKATMTVDTSTNTAYMELSSLRSEDTAVYYCASRDYDYDGRYFDYWGQGTLVTVSSASTKGPSVFPLAPSSKSTSGGTAALGCLVKDYFPEPVTVSWNSGALTSGVHTFPAVLQSSGLYSLSSVVTVPSSSLGTQTYICNVNHKPSNTKVDEKVEPKSCDKTHTCPPCPAPELLGGPSVFLFPPKPKDTLMISRTPEVTCVVVDVSHEDPEVKFNWYVDGVEVHNAKTKPREEQYQSTYRVVSVLTVLHQDWLNGKEYKCKVSNKALPAPIEKTISKAKGQPRRPRVYTLPPSREEMTKNQVSLVCLVKGFYPSDIAVEWESNGQPENNYKTTPPVLDSDGSFFLYSVLTVDKSRWQQGNVFSCSVMHEALHNHYTQKSLSLSPG

SEQ ID NO: 48 - protein, 213 aa, Artificial Sequence
  Synthetic Construct
DIQMTQSPSSLSASVGDRVTITCSASSSVTYMYWYQQKPGKAPKLLIYDTSNLASGVPSRFSGSGSGTDYTFTISSLQPEDIATYYCQQWSSHIFTFGQGTKVEIKRTVAAPSVFIFPPSDEQLKSGTASVVCLLNNFYPREAKVQWKVDNALQSGNSQESVTEQDSKDSTYSLSSTLTLSKADYEKHKVYACEVTHQGLSSPVTKSFNRGEC

SEQ ID NO: 49 - protein, 213 aa, Artificial Sequence
  Synthetic Construct
DIQMTQSPSSLSASVGDRVTITCSASSSVTYMYWYQQKPGKAPKLLIYDTSNLASGVPSRFSGSGSGTDYTFTISSLQPEDIATYYCQQWSSHIFTFGQGTKVEIKRTVAAPSVFIFPPSDKQLKSGTASVVCLLNNFYPREAKVQWKVDNALQSGNSQESVTEQDSKDSTYSLSSTLTLSKADYEKHKVYACEVTHQGLSSPVTKSFNRGEC

SEQ ID NO: 50 - protein, 445 aa, Artificial Sequence
  Synthetic Construct
QVQLVQSGAEVKKPGSSVKVSCKASGYTFTTYYLHWVRQAPGQGLEWMGWIYPGNVHAQYNEKFKGRVTITADKSTSTAYMELSSLRSEDTAVYYCARSWEGFPYWGQGTTVTVSSASTKGPSVFPLAPSSKSTSGGTAALGCLVKDYFPEPVTVSWNSGALTSGVHTFPAVLQSSGLYSLSSVVTVPSSSLGTQTYICNVNHKPSNTKVDKKVEPKSCDKTHTCPPCPAPELLGGPSVFLFPPKPKDTLMISRTPEVTCVVVDVSHEDPEVKFNWYVDGVEVHNAKTKPREEQYQSTYRVVSVLTVLHQDWLNGKEYKCKVSNKALPAPIEKTISKAKGQPRRPRVYTLPPSREEMTKNQVSLVCLVKGFYPSDIAVEWESNGQPENNYKTTPPVLDSDGSFFLYSVLTVDKSRWQQGNVFSCSVMHEALHNHYTQKSLSLSPG

SEQ ID NO: 51 - protein, 445 aa, Artificial Sequence
  Synthetic Construct
QVQLVQSGAEVKKPGSSVKVSCKASGYTFTTYYLHWVRQAPGQGLEWMGWIYPGNVHAQYNEKFKGRVTITADKSTSTAYMELSSLRSEDTAVYYCARSWEGFPYWGQGTTVTVSSASTKGPSVFPLAPSSKSTSGGTAALGCLVKDYFPEPVTVSWNSGALTSGVHTFPAVLQSSGLYSLSSVVTVPSSSLGTQTYICNVNHKPSNTKVDEKVEPKSCDKTHTCPPCPAPELLGGPSVFLFPPKPKDTLMISRTPEVTCVVVDVSHEDPEVKFNWYVDGVEVHNAKTKPREEQYQSTYRVVSVLTVLHQDWLNGKEYKCKVSNKALPAPIEKTISKAKGQPRRPRVYTLPPSREEMTKNQVSLVCLVKGFYPSDIAVEWESNGQPENNYKTTPPVLDSDGSFFLYSVLTVDKSRWQQGNVFSCSVMHEALHNHYTQKSLSLSPG

SEQ ID NO: 52 - protein, 214 aa, Artificial Sequence
  Synthetic Construct
DIQMTQSPSSLSASVGDRVTITCKASQNVGINVAWYQQKPGKAPKSLISSASYRYSGVPSRFSGSGSGTDFTLTISSLQPEDFATYFCQQYDTYPFTFGQGTKVEIKRTVAAPSVFIFPPSDEQLKSGTASVVCLLNNFYPREAKVQWKVDNALQSGNSQESVTEQDSKDSTYSLSSTLTLSKADYEKHKVYACEVTHQGLSSPVTKSFNRGEC

SEQ ID NO: 53 - protein, 214 aa, Artificial Sequence
  Synthetic Construct
DIQMTQSPSSLSASVGDRVTITCKASQNVGINVAWYQQKPGKAPKSLISSASYRYSGVPSRFSGSGSGTDFTLTISSLQPEDFATYFCQQYDTYPFTFGQGTKVEIKRTVAAPSVFIFPPSDKQLKSGTASVVCLLNNFYPREAKVQWKVDNALQSGNSQESVTEQDSKDSTYSLSSTLTLSKADYEKHKVYACEVTHQGLSSPVTKSFNRGEC

SEQ ID NO: 54 - protein, 337 aa, Artificial Sequence; identical to SEQ ID NO: 1
  Synthetic Construct

SEQ ID NO: 55 - protein, 107 aa, Artificial Sequence [sequence omitted]

SEQ ID NO: 56 - protein, 337 aa, Artificial Sequence
  Synthetic Construct
ASTKGPSVFPLAPSSKSTSGGTAALGCLVADYFPEPVTVSWNSGALTSGVHTFPAVLQSSGLYSLSSVVTVPSSSLGTQTYICNVNHKPSNTKVDEKVEPKSCDKGSIEGRGSTHTCPPCPAPELLGGPSVFLFPPKPKDTLMISRTPEVTCVVVDVSHEDPEVKFNWYVDGVEVHNAKTKPREEQYNSTYRVVSVLTVLHQDWLNGKEYKCKVSNKALPAPIEKTISKAKGQPREPQVYTLPPSRDELTKNQVSLTCLVKGFYPSDIAVEWESNGQPENNYKTTPPVLDSDGSFFLYSKLTVDKSRWQQGNVFSCSVMHEALHNHYTQKSLSLSPG

SEQ ID NO: 57 - protein, 107 aa, Artificial Sequence
  Synthetic Construct
RTVAAPSVFIFPPSDKQLKSGTARVVCLLNNFYPREAKVQWKVDNALQSGNSQESVTEQDSKDSTYSLSSTLTLSKADYEKHKVYACEVTHQGLSSPVTKSFNRGEC

SEQ ID NO: 58 - protein, 337 aa, Artificial Sequence
  Synthetic Construct
ASTKGPSVFPLAPSSKSTSGGTAALGCLVADYFPEPVTVSWNSGALTSGVHTFPAVLQSSGLYSLASVVTVPSSSLGTQTYICNVNHKPSNTKVDKKVEPKSCDKGSIEGRGSTHTCPPCPAPELLGGPSVFLFPPKPKDTLMISRTPEVTCVVVDVSHEDPEVKFNWYVDGVEVHNAKTKPREEQYNSTYRVVSVLTVLHQDWLNGKEYKCKVSNKALPAPIEKTISKAKGQPREPQVYTLPPSRDELTKNQVSLTCLVKGFYPSDIAVEWESNGQPENNYKTTPPVLDSDGSFFLYSKLTVDKSRWQQGNVFSCSVMHEALHNHYTQKSLSLSPG

SEQ ID NO: 59 - protein, 107 aa, Artificial Sequence
  Synthetic Construct
RTVAAPSVFIFPPSDEQLKSGTARVVCLLNNFYPREAKVQWKVDNALQSGNSQESVTEQDSKDSTYSLISTLTLSKADYEKHKVYACEVTHQGLSSPVTKSFNRGEC

SEQ ID NO: 60 - protein, 337 aa, Artificial Sequence
  Synthetic Construct
ASTKGPSVFPLAPSSKSTSGGTAALGCLVKDYFPEPVTVSWNSGALTSGVHTFPAVLQSSGLYSLSSVVTVPSSSLGTQTYICNVNHKPSNTKVDEKVEPKSCDKGSIEGRGSTHTCPPCPAPELLGGPSVFLFPPKPKDTLMISRTPEVTCVVVDVSHEDPEVKFNWYVDGVEVHNAKTKPREEQYNSTYRVVSVLTVLHQDWLNGKEYKCKVSNKALPAPIEKTISKAKGQPREPQVYTLPPSRDELTKNQVSLTCLVKGFYPSDIAVEWESNGQPENNYKTTPPVLDSDGSFFLYSKLTVDKSRWQQGNVFSCSVMHEALHNHYTQKSLSLSPG

SEQ ID NO: 61 - protein, 107 aa, Artificial Sequence
  Synthetic Construct
RTVAAPSVFIFPPSDKQLKSGTASVVCLLNNFYPREAKVQWKVDNALQSGNSQESVTEQDSKDSTYSLSSTLTLSKADYEKHKVYACEVTHQGLSSPVTKSFNRGEC

SEQ ID NO: 62 - protein, 337 aa, Artificial Sequence
  Synthetic Construct
ASTKGPSVFPLAPSSKSTSGGTAALGCLVADYFPEPVTVSWNSGALTSGVHTFPAVLQSSGLYSLGSVVTVPSSSLGTQTYICNVNHKPSNTKVDKKVEPKSCDKGSIEGRGSTHTCPPCPAPELLGGPSVFLFPPKPKDTLMISRTPEVTCVVVDVSHEDPEVKFNWYVDGVEVHNAKTKPREEQYNSTYRVVSVLTVLHQDWLNGKEYKCKVSNKALPAPIEKTISKAKGQPREPQVYTLPPSRDELTKNQVSLTCLVKGFYPSDIAVEWESNGQPENNYKTTPPVLDSDGSFFLYSKLTVDKSRWQQGNVFSCSVMHEALHNHYTQKSLSLSPG

SEQ ID NO: 63 - protein, 337 aa, Artificial Sequence
  Synthetic Construct
ASTKGPSVFPLAPSSKSTSGGTAALGCLVADYFPEPVTVSWNSGALTSGVHTFPAVLQSSGLYSLASVVTVPSSSLGTQTYICNVNHKPSNTKVDEKVEPKSCDKGSIEGRGSTHTCPPCPAPELLGGPSVFLFPPKPKDTLMISRTPEVTCVVVDVSHEDPEVKFNWYVDGVEVHNAKTKPREEQYNSTYRVVSVLTVLHQDWLNGKEYKCKVSNKALPAPIEKTISKAKGQPREPQVYTLPPSRDELTKNQVSLTCLVKGFYPSDIAVEWESNGQPENNYKTTPPVLDSDGSFFLYSKLTVDKSRWQQGNVFSCSVMHEALHNHYTQKSLSLSPG

SEQ ID NO: 64 - protein, 107 aa, Artificial Sequence
  Synthetic Construct
RTVAAPSVFIFPPSDKQLKSGTARVVCLLNNFYPREAKVQWKVDNALQSGNSQESVTEQDSKDSTYSLISTLTLSKADYEKHKVYACEVTHQGLSSPVTKSFNRGEC

SEQ ID NO: 65 - protein, 337 aa, Artificial Sequence
  Synthetic Construct
ASTKGPSVFPLAPSSKSTSGGTAALGCLVADYFPEPVTVSWNSGALTSGVHTFPAVLQSSGLYSLGSVVTVPSSSLGTQTYICNVNHKPSNTKVDEKVEPKSCDKGSIEGRGSTHTCPPCPAPELLGGPSVFLFPPKPKDTLMISRTPEVTCVVVDVSHEDPEVKFNWYVDGVEVHNAKTKPREEQYNSTYRVVSVLTVLHQDWLNGKEYKCKVSNKALPAPIEKTISKAKGQPREPQVYTLPPSRDELTKNQVSLTCLVKGFYPSDIAVEWESNGQPENNYKTTPPVLDSDGSFFLYSKLTVDKSRWQQGNVFSCSVMHEALHNHYTQKSLSLSPG

SEQ ID NO: 66 - protein, 98 aa, Artificial Sequence
  Synthetic Construct
ASTKGPSVFPLAPSSKSTSGGTAALGCLVKDYFPEPVTVSWNSGALTSGVHTFPAVLQSSGLYSLSSVVTVPSSSLGTQTYICNVNHKPSNTKVDKKV

SEQ ID NO: 67 - protein, 98 aa, Artificial Sequence
  Synthetic Construct
ASTKGPSVFPLAPSSKSTSGGTAALGCLVADYFPEPVTVSWNSGALTSGVHTFPAVLQSSGLYSLSSVVTVPSSSLGTQTYICNVNHKPSNTKVDEKV

SEQ ID NO: 68 - protein, 98 aa, Artificial Sequence
  Synthetic Construct
ASTKGPSVFPLAPSSKSTSGGTAALGCLVADYFPEPVTVSWNSGALTSGVHTFPAVLQSSGLYSLASVVTVPSSSLGTQTYICNVNHKPSNTKVDKKV

SEQ ID NO: 69 - protein, 98 aa, Artificial Sequence
  Synthetic Construct
ASTKGPSVFPLAPSSKSTSGGTAALGCLVKDYFPEPVTVSWNSGALTSGVHTFPAVLQSSGLYSLSSVVTVPSSSLGTQTYICNVNHKPSNTKVDEKV

SEQ ID NO: 70 - protein, 98 aa, Artificial Sequence
  Synthetic Construct
ASTKGPSVFPLAPSSKSTSGGTAALGCLVADYFPEPVTVSWNSGALTSGVHTFPAVLQSSGLYSLGSVVTVPSSSLGTQTYICNVNHKPSNTKVDKKV

SEQ ID NO: 71 - protein, 98 aa, Artificial Sequence
  Synthetic Construct
ASTKGPSVFPLAPSSKSTSGGTAALGCLVADYFPEPVTVSWNSGALTSGVHTFPAVLQSSGLYSLASVVTVPSSSLGTQTYICNVNHKPSNTKVDEKV

SEQ ID NO: 72 - protein, 98 aa, Artificial Sequence
  Synthetic Construct
ASTKGPSVFPLAPSSKSTSGGTAALGCLVADYFPEPVTVSWNSGALTSGVHTFPAVLQSSGLYSLGSVVTVPSSSLGTQTYICNVNHKPSNTKVDEKV

SEQ ID NO: 73 - protein, 217 aa, Artificial Sequence
  Synthetic Construct
APELLGGPSVFLFPPKPKDTLMISRTPEVTCVVVDVSHEDPEVKFNWYVDGVEVHNAKTKPREEQYNSTYRVVSVLTVLHQDWLNGKEYKCKVSNKALPAPIEKTISKAKGQPREPQVYTLPPSREEMTKNQVSLTCLVKGFYPSDIAVEWESNGQPENNYKTTPPVLDSDGSFFLYSKLTVDKSRWQQGNVFSCSVMHEALHNHYTQKSLSLSPGK

SEQ ID NO: 74 - protein, 217 aa, Artificial Sequence
  Synthetic Construct
APELLGGPSVFLFPPKPKDTLMISRTPEVTCVVVDVSHEDPEVKFNWYVDGVEVHNAKTKPREEQYNSTYRVVSVLTVLHQDWLNGKEYKCKVSNKALPAPIEKTISKAKGQPREPQVYTLPPSREEMTKNQVSLTCLVKGFYPSDIAVEWESNGQPENNYKTTPPVLMSDGSFFLASKLTVDKSRWQQGNVFSCSVMHEALHNHYTQKSLSLSPGK

SEQ ID NO: 75 - protein, 217 aa, Artificial Sequence
  Synthetic Construct
APELLGGPSVFLFPPKPKDTLMISRTPEVTCVVVDVSHEDPEVKFNWYVDGVEVHNAKTKPREEQYNSTYRVVSVLTVLHQDWLNGKEYKCKVSNKALPAPIEKTISKAKGQPREPQVYTLPPSREEMTDNQVSLTCLVKGFYPSDIAVEWESNGQPENNYKTTPPVLMSDGSFFLASKLTVDKSRWQQGNVFSCSVMHEALHNHYTQKSLSLSPGK

SEQ ID NO: 76 - protein, 217 aa, Artificial Sequence
  Synthetic Construct
APELLGGPSVFLFPPKPKDTLMISRTPEVTCVVVDVSHEDPEVKFNWYVDGVEVHNAKTKPREEQYNSTYRVVSVLTVLHQDWLNGKEYKCKVSNKALPAPIEKTISKAKGQPREPQVSTLPPSREEMTKNQVSLVCLVYGFYPSDIAVEWESNGQPENNYKTTPPVLDSDGSFFLYSVLTVDKSRWQQGNVFSCSVMHEALHNHYTQKSLSLSPGK

SEQ ID NO: 77 - protein, 217 aa, Artificial Sequence
  Synthetic Construct
APELLGGPSVFLFPPKPKDTLMISRTPEVTCVVVDVSHEDPEVKFNWYVDGVEVHNAKTKPREEQYNSTYRVVSVLTVLHQDWLNGKEYKCKVSNKALPAPIEKTISKAKGQPREPQVSTLPPSREEMTKNQVSLMCLVYGFYPSDIAVEWESNGQPENNYKTTPPVLDSDGSFFLYSVLTVDKSRWQQGNVFSCSVMHEALHNHYTQKSLSLSPGK

SEQ ID NO: 78 - protein, 217 aa, Artificial Sequence
  Synthetic Construct
APELLGGPSVFLFPPKPKDTLMISRTPEVTCVVVDVSHEDPEVKFNWYVDGVEVHNAKTKPREEQYNSTYRVVSVLTVLHQDWLNGKEYKCKVSNKALPAPIEKTISKAKGQPREPQVYTLPPSREEMTKNQVSLVCLVKGFYPSDIAVEWESNGQPENNYKTTPPVLDSDGSFFLYSVLTVDKSRWQQGNVFSCSVMHEALHNHYTQKSLSLSPGK

SEQ ID NO: 79 - protein, 217 aa, Artificial Sequence
  Synthetic Construct
APELLGGPSVFLFPPKPKDTLMISRTPEVTCVVVDVSHEDPEVKFNWYVDGVEVHNAKTKPREEQYNSTYRVVSVLTVLHQDWLNGKEYKCKVSNKALPAPIEKTISKAKGQPRRPRVYTLPPSREEMTKNQVSLVCLVKGFYPSDIAVEWESNGQPENNYKTTPPVLDSDGSFFLYSVLTVDKSRWQQGNVFSCSVMHEALHNHYTQKSLSLSPGK

SEQ ID NO: 80 - protein, 217 aa, Artificial Sequence
  Synthetic Construct
APELLGGPSVFLFPPKPKDTLMISRTPEVTCVVVDVSHEDPEVKFNWYVDGVEVHNAKTKPREEQYNSTYRVVSVLTVLHQDWLNGKEYKCKVSNKALPAPIEKTISKAKGQPREPQVYTLPPSREDMTKNQVQLTCLVKGFYPSDIAVEWESNGQPENNYKTTPPVLDSDGSFFLASKLTVDKSRWQQGNVFSCSVMHEALHNHYTQKSLSLSPGK

SEQ ID NO: 81 - protein, 217 aa, Artificial Sequence
  Synthetic Construct
APELLGGPSVFLFPPKPKDTLMISRTPEVTCVVVDVSHEDPEVKFNWYVDGVEVHNAKTKPREEQYNSTYRVVSVLTVLHQDWLNGKEYKCKVSNKALPAPIEKTISKAKGQPREPQVYTLPPSRGDMTKNQVQLTCLVKGFYPSDIAVEWESNGQPENNYKTTPPVLDSDGSFFLASKLTVDKSRWQQGNVFSCSVMHEALHNHYTQKSLSLSPGK

SEQ ID NO: 82 - protein, 217 aa, Artificial Sequence
  Synthetic Construct
APELLGGPSVFLFPPKPKDTLMISRTPEVTCVVVDVSHEDPEVKFNWYVDGVEVHNAKTKPREEQYNSTYRVVSVLTVLHQDWLNGKEYKCKVSNKALPAPIEKTISKAKGQPREPQVYTLPPSREDMTKNQVRLTCLVKGFYPSDIAVEWESNGQPENNYKTTPPVLDSDGSFFLASKLTVDKSRWQQGNVFSCSVMHEALHNHYTQKSLSLSPGK

SEQ ID NO: 83 - protein, 217 aa, Artificial Sequence
  Synthetic Construct
APELLGGPSVFLFPPKPKDTLMISRTPEVTCVVVDVSHEDPEVKFNWYVDGVEVHNAKTKPREEQYNSTYRVVSVLTVLHQDWLNGKEYKCKVSNKALPAPIEKTISKAKGQPREPQVYTLPPSREEMTKNQVSLTCLVKGFYPSDIAVEWESNGQPENNYKTTPPVLDSDGSFFLASKLTVDKSRWQQGNVFSCSVMHEALHNHYTQKSLSLSPGK

SEQ ID NO: 84 - protein, 217 aa, Artificial Sequence
  Synthetic Construct
APELLGGPSVFLFPPKPKDTLMISRTPEVTCVVVDVSHEDPEVKFNWYVDGVEVHNAKTKPREEQYNSTYRVVSVLTVLHQDWLNGKEYKCKVSNKALPAPIEKTISKAKGQPREPQVYTLPPSREEMTKNQVSLMCLVKGFYPSDIAVEWESNGQPENNYKTTPPVLDSDGSFFLYSVLTVDKSRWQQGNVFSCSVMHEALHNHYTQKSLSLSPGK